European Patent Specification EP 3 688 197 B1, published May 14, 2025. Title: NEW LACTOBACILLUS PLANTARUM STRAIN AND USES THEREOF. Applicant: DuPont Nutrition Biosciences ApS. The sequence listing filed with the application follows.

SEQUENCE LISTING (7 sequences)

SEQ ID NO: 1 - DNA, 6453 bp, Lactobacillus plantarum
gtgggtgatccagttcctacagtcaaattccttggactgacgtttaatatcgcgaatgacatctcagtaattgtgacttgtctgattgttttcttgtttgtttttttactttcgcgacatttaacaatgaagcccaagggtggacaaaatgtgctggagtggctcatcgagttcacgaatggcattgtcaaagggtcgatcaagggtaacgaagcgtctaacttcggtttgtacgcatttacattgtttctctttatcttcatcgctaaccaacttggattgttcattcacgttcaggtcgggcagtatacgtatctgaagagtccaaccgccgatccgattgtgactttgacgttatcgtttatgaccgttgcacttgcacatgctgcgggtgttcgtaagaaaggtatgggtggttatttgaaagaatacacacaaccttttgctgttttctcggttgttaacgtctttgaacaatttaccgatttcctaactttaggtcttcggctgttcgggaacatctttgctggtgaaatgttactaacgaaggttgctgatttggcaaagagcaacggttggttgagctatgtttactcatttccaattgaactcttatggcaaggtttctcagtgtttatcgggagcattcaagcgttcgtgttcgtaaccttgacttcagtttatatttctcagaaggttaacgacgaggaataatttctagttttttaattttaaggaggatacacagattatgggagcaattgctgcaggtattgctatgtgtggtgccgctataggtgctggtattggtaacggtttggttatttctaagatgcttgaagggatggcccgtcaaccagaattatctggtcaattacggactaacatgttcatcggtgttgggttggtcgaatcaatgcctataatttccttcgttgttgctttgatggttatgaacaagtaatcattggtcaacgagttcattttaatgaaaatgaaagaaggaggtgtcattagatgctctcgcatttaattatcggtgcatccggtctctaccttggtgatatgttgtttatcgggattagctttattgttttgatggcattgatctctgttgttgcttggaagcccatcacaaaaatgatggctgatcgagccgacaagattgcgaacgacattgattcagcacaaaagtctcggcaagaagcgagtgacttagctgatcaacggcgtgatgcgctatcacactctcgcgctgaagcgagtgaaattgtcgctgacgcgaaaaagagtggcgaaaagcaacggtcaagtatcattgccgatgcgcaaaacgaagcaacgcagtataaacaaaatgcgcgtaaggatattgaacaggagcgtcaagatgccttgaagaacgtccaatcagacgtcgctgacatttcgattgcgattgctacgaagattattaagaagcaattggatccggaaggccaacaggcattaattaattcgtatattgaagggttgggaaagcatgagtcttgataatcttacaattgcaagtcgttattcaaaggcactctttgaacttgcagttgaaaaagatcagaccgaagcattcctggccgagttaaagcaattacggcaagtctttgtcgacaacccgcaattggcagaggtcctctcaggatcattgcttccggttgatcaaaaacagacaacgttgtcaactttgactgaccacgcttcagaatacattaaaaactttattcaaatgttgtatgattacggccgcatgtcgaacttagttggcattgttgacgcgtttgaagcacgtttcgatgagagtcgcaaaatagtgcatgccgaagtaacgtctgcggtcaagttgtcagatgagcaagctgatgcaatcgcaaaggcattcgccaaacgtgttggggccaatcaggttgttttgtcacgtaaagtcgatgaagcaatcattggcggtgtaattgtgaagtcaaataatcaaacgtttgatggtagcgttgcgttacaactaacgaatttaagacgagcactcatcaacaattagtttacgaagaggtgaaacttttatgagcattaaatctgaagaaatcagtgctctaatcaaacaacaattagaaagttatcaaactgagctctcagttgctgaaaccggtactgtcacctacgttggtgatgggatcgcccgtgctcacggactcgacaacgccttacaaggtgaattactcgaattcagtaacggagtttacgggatggtacaaaacctcgaaagcaacgatgttggtatcgttgttttaggggattttgatggtattcgtgaaggcgatactgttaagcggactggccgcatcatggaagttccagtcggtgacgccatgattggccgggtcgttaacccattaggtcaaccagttgacggttcaggtgagattaagaccacgaatacgcggccaatcgaacataaagctcctggtattatgcaacggcaatcagttagcgaaccacttcaaactgggatcaaggccattgatgccttagttccaattggtcggggccaacgtgaattgattatcggtgaccgtaagactgggaagacgtccgttgccattgatgccattttgaaccaaaaggaccaagacatgatttgtgtctacgttgcaatcggtcaaaaggactcaactgtacgggcccaagttgaaacgttgaagaagttaggtgcgatggactacacaatcgttgtaactgccggacctgctgaaccagcgccattactgtacttagctccttatgctggggcagcgatgggtgaagaatttatgatgaacggcaagcacgttttgatcgtctatgatgacctttcaaagcaagcaacggcttaccgtgaactttccttgatcctccgtcgtcctccaggtcgtgaagcttatcctggggatgtcttctacttgcactcacggttactcgaacgggctgccaagttgagcgatgaattgggtggcggttcaatgacggccttaccaattatcgaaacgcaagctggggatatttcggcttatattccaactaacgttatttcaatcaccgatgggcaaatcttcttggatagtgattcattctattcaggtgtgcggccagcgattgatgccggggcctctgtttcccgggttggtggggatgcgcaaattaaagcgatgaagtccgttgccgggaccttgcgtcttgacttggcttcttatcgtgaattggaatccttctcacaattcggttctgacttggatgctgcaacccaagcgaaattaaatcgtgggcaacggatcgttgaagtcttaaaacaacctgttcattcaccattgaaggtcgaagaacaagtaatgattttatatgctttgaccaacggttatttggataaagtggcagttgatgatattgcccgttaccaaagtgaattgtttgaatttattcatgctagtcatcaggacctctttgatacgattttggcaaccaagaagttaccagaagctgataagatgaatggggccttagatgcgtttgcagaacaattccagccaaccgctgccgctgcgaagtagttatggctgaaaaggatggtgagtagtgcatggcagaatcattaatggatgtcaagcgccgaattgactcaacaaagaagactcatcaaattacgtcggcaatgcaaatggtctcaacttcaaaattgaaccagattcaaaagcataccagcacgtatcaggtgtacgcttctaaagttgaaagcatcgtttcacatcttgccaaagctcatctgatgtcagcaagtgccggtgttgctaacagtaattcgaacacgatttcagttagtgaattgctcgcgcaacgccccgttaaaaagactggtttattggtgatcacttcggaccgtggcctcgttggtagttacaacagtaacgtgttgaaacagactaacgatttcatgcggacgcacaaggttgatgccgataacgcagtcgttttggcggttggtggcactggtgcggatttctataaaaagaacgggttaaacgtggcttatgagtaccgcggcgtctctgatgtcccaacttttaaagaggttcgtgaaatcgttaagacagtcacatcaatgtaccacaacgaagtctttgatgaactttacgtcttctacaaccactttattaatcggctctcttctggttttcgggccgttaagatgttaccgatctccgaagagacctttgaacaaagtgagtcagataatcgtaaagccaaggatagccgggtagatgtcggtcccgagtatgaaatggaaccgtcagaagaagccattttgtcggccgtgttgccacaatatgctgaaagcttggtttatggtgcaatcttggatgccaagactgctgaacatgcttcgtcgtcaaccgcgatgaaggctgcatcagataacgctggcgatttaatcgataaattaaatctgaaatataaccgtgcgcgtcaagctgctattaccactgaaatcactgaaatcactggtggtttggttgcgcaagaataacgaagtgggaggaattaacgactaatgagtacaggtaaagttgtacaagttattggacccgttgttgacgttgaattctctctaaacgataagttacccgatattaataacgccttgatcattcagaaggacaacgatgacactttaacggtggaagtatcgttggaattaggtgatggggttgttcggaccgtcgcgatggatggtacggatggcttgcgccggggaatgacagttgaagacactggttcttcaattactgttcccgttggtaaagagacgttaggccgggtcttcaacgttttaggggaaaccattgatggtggtccagaattcggtccagacgcagaacgtaacccgattcatcgggatgcgcctaaatatgatgaattaacgaccagtactgaagtattggaaactggaattaaagttattgacctcttagcaccttatgttcgtggtggtaagattgggttgttcggtggtgccggtgttggtaaaactgttttaatccaggaattaattcataacattgcccaagaacataacgggatttccgtgtttaccggtgttggtgaacggacgcgtgaagggaatgacctttacttcgaaatgaaggcttccggcgttttgaagaataccgccatggtttatggtcaaatgaacgaaccacctggtgcccggatgcgggtggccttgaccggtttgacgattgcggaatacttccgtgatgttcaaggtcaagacgtgttgttattcatcgacaatatcttccggttcacgcaagctggttctgaagtttccgccttacttggtcggattccttcagccgttggttaccaaccaaccttagccactgaaatgggtcaattacaagaacggatcacttctaccaagaaggggtcagttacttcgattcaagccgtttatgtacctgccgatgattataccgacccggcacctgcaacgactttcgcccatttggatgcgacgaccaacttggaacgttctttgacggaacaagggatctacccagccgttgacccattagcttcttcttcaatcgctctggacccatcaatcgtgggcgaagaacattatcaagttgcaacggaagttcaacgggtcttgcaacgttatcgtgaattgcaagatattatctcgattttagggatggatgaattatctgacgaagaaaagacaactgttgcgcgtgcacggcggattcaattcttcttgtcacaaaacttcttcgttgccgaaaactttacgggccaacctggttcgtatgtgccaatcaacgataccatcaagggcttcaaagaaattcttgaaggtaaatatgatgacctaccagaagacgcattccgtcaagttggtaagatcgacgacgtggtcgaaaaagcgaaatcgatggtaactgattaggaggggtttacatggctgacaatgcaaaatcattaaccgttagcatcgtaactccagacggtcaggtctatgagaataagacgccaatgttgatcgtgcgaacgattgacggcgaactcggaattttgccgaaccatattcctgtgattgcatcgcttgcaatcgatgaggttcggatcaagcaacttgaaagtgatcaggaagatgacgaaattgccgttaatggtggttttgttgagttcagtaataatacggcaacgattgttgccgatagtgctgaacgtcagaatgacattgacgttgctcgagctgaaaatgcacggaaacgcgctgaaacacggattcaaaatgcccaacaaaagcacgatgatgctgagttggcgcgggcccaagtcgctttgcggcgtgccatgaaccgtttgaatgttgctcggcattaa

SEQ ID NO: 2 - DNA, 1521 bp, Lactobacillus plantarum
atgagcattaaatctgaagaaatcagtgctctaatcaaacaacaattagaaagttatcaaactgagctctcagttgctgaaaccggtactgtcacctacgttggtgatgggatcgcccgtgctcacggactcgacaacgccttacaaggtgaattactcgaattcagtaacggagtttacgggatggtacaaaacctcgaaagcaacgatgttggtatcgttgttttaggggattttgatggtattcgtgaaggcgatactgttaagcggactggccgcatcatggaagttccagtcggtgacgccatgattggccgggtcgttaacccattaggtcaaccagttgacggttcaggtgagattaagaccacgaatacgcggccaatcgaacataaagctcctggtattatgcaacggcaatcagttagcgaaccacttcaaactgggatcaaggccattgatgccttagttccaattggtcggggccaacgtgaattgattatcggtgaccgtaagactgggaagacgtccgttgccattgatgccattttgaaccaaaaggaccaagacatgatttgtgtctacgttgcaatcggtcaaaaggactcaactgtacgggcccaagttgaaacgttgaagaagttaggtgcgatggactacacaatcgttgtaactgccggacctgctgaaccagcgccattactgtacttagctccttatgctggggcagcgatgggtgaagaatttatgatgaacggcaagcacgttttgatcgtctatgatgacctttcaaagcaagcaacggcttaccgtgaactttccttgatcctccgtcgtcctccaggtcgtgaagcttatcctggggatgtcttctacttgcactcacggttactcgaacgggctgccaagttgagcgatgaattgggtggcggttcaatgacggccttaccaattatcgaaacgcaagctggggatatttcggcttatattccaactaacgttatttcaatcaccgatgggcaaatcttcttggatagtgattcattctattcaggtgtgcggccagcgattgatgccggggcctctgtttcccgggttggtggggatgcgcaaattaaagcgatgaagtccgttgccgggaccttgcgtcttgacttggcttcttatcgtgaattggaatccttctcacaattcggttctgacttggatgctgcaacccaagcgaaattaaatcgtgggcaacggatcgttgaagtcttaaaacaacctgttcattcaccattgaaggtcgaagaacaagtaatgattttatatgctttgaccaacggttatttggataaagtggcagttgatgatattgcccgttaccaaagtgaattgtttgaatttattcatgctagtcatcaggacctctttgatacgattttggcaaccaagaagttaccagaagctgataagatgaatggggccttagatgcgtttgcagaacaattccagccaaccgctgccgctgcgaagtag

SEQ ID NO: 3 - protein, 506 aa, Lactobacillus plantarum
MSIKSEEISALIKQQLESYQTELSVAETGTVTYVGDGIARAHGLDNALQGELLEFSNGVYGMVQNLESNDVGIVVLGDFDGIREGDTVKRTGRIMEVPVGDAMIGRVVNPLGQPVDGSGEIKTTNTRPIEHKAPGIMQRQSVSEPLQTGIKAIDALVPIGRGQRELIIGDRKTGKTSVAIDAILNQKDQDMICVYVAIGQKDSTVRAQVETLKKLGAMDYTIVVTAGPAEPAPLLYLAPYAGAAMGEEFMMNGKHVLIVYDDLSKQATAYRELSLILRRPPGREAYPGDVFYLHSRLLERAAKLSDELGGGSMTALPIIETQAGDISAYIPTNVISITDGQIFLDSDSFYSGVRPAIDAGASVSRVGGDAQIKAMKSVAGTLRLDLASYRELESFSQFGSDLDAATQAKLNRGQRIVEVLKQPVHSPLKVEEQVMILYALTNGYLDKVAVDDIARYQSELFEFIHASHQDLFDTILATKKLPEADKMNGALDAFAEQFQPTAAAAK

SEQ ID NO: 4 - DNA, 1521 bp, Lactobacillus plantarum
atgagcattaaatctgaagaaatcagtgctctaatcaaacaacaattagaaagttatcaaactgagctctcagttgctgaaaccggtactgtcacctacgttggtgatgggatcgcccgtgctcacggactcgacaacgccttacaaggtgaattactcgaattcagtaacggagtttacgggatggtacaaaacctcgaaagcaacgatgttggtatcgttgttttaggggattttgatggtattcgtgaaggcgatactgttaagcggactggccgcatcatggaagttccagtcggtgacgccatgattggccgggtcgttaacccattaggtcaaccagttgacggttcaggtgagattaagaccacgaatacgcggccaatcgaacataaagctcctggtattatgcaacggcaatcagttagcgaaccacttcaaactgggatcaaggccattgatgccttagttccaattggtcggggccaacgtgaattgattatcgatgaccgtaagactgggaagacgtccgttgccattgatgccattttgaaccaaaaggaccaagacatgatttgtgtctacgttgcaatcggtcaaaaggactcaactgtacgggcccaagttgaaacgttgaagaagttaggtgcgatggactacacaatcgttgtaactgccggacctgctgaaccagcgccattactgtacttagctccttatgctggggcagcgatgggtgaagaatttatgatgaacggcaagcacgttttgatcgtctatgatgacctttcaaagcaagcaacggcttaccgtgaactttccttgatcctccgtcgtcctccaggtcgtgaagcttatcctggggatgtcttctacttgcactcacggttactcgaacgggctgccaagttgagcgatgaattgggtggcggttcaatgacggccttaccaattatcgaaacgcaagctggggatatttcggcttatattccaactaacgttatttcaatcaccgatgggcaaatcttcttggatagtgattcattctattcaggtgtgcggccagcgattgatgccggggcctctgtttcccgggttggtggggatgcgcaaattaaagcgatgaagtccgttgccgggaccttgcgtcttgacttggcttcttatcgtgaattggaatccttctcacaattcggttctgacttggatgctgcaacccaagcgaaattaaatcgtgggcaacggatcgttgaagtcttaaaacaacctgttcattcaccattgaaggtcgaagaacaagtaatgattttatatgctttgaccaacggttatttggataaagtggcagttgatgatattgcccgttaccaaagtgaattgtttgaatttattcatgctagtcatcaggacctctttgatacgattttggcaaccaagaagttaccagaagctgataagatgaatggggccttagatgcgtttgcagaacaattccagccaaccgctgccgctgcgaagtag

SEQ ID NO: 5 - protein, 506 aa, Lactobacillus plantarum
MSIKSEEISALIKQQLESYQTELSVAETGTVTYVGDGIARAHGLDNALQGELLEFSNGVYGMVQNLESNDVGIVVLGDFDGIREGDTVKRTGRIMEVPVGDAMIGRVVNPLGQPVDGSGEIKTTNTRPIEHKAPGIMQRQSVSEPLQTGIKAIDALVPIGRGQRELIIDDRKTGKTSVAIDAILNQKDQDMICVYVAIGQKDSTVRAQVETLKKLGAMDYTIVVTAGPAEPAPLLYLAPYAGAAMGEEFMMNGKHVLIVYDDLSKQATAYRELSLILRRPPGREAYPGDVFYLHSRLLERAAKLSDELGGGSMTALPIIETQAGDISAYIPTNVISITDGQIFLDSDSFYSGVRPAIDAGASVSRVGGDAQIKAMKSVAGTLRLDLASYRELESFSQFGSDLDAATQAKLNRGQRIVEVLKQPVHSPLKVEEQVMILYALTNGYLDKVAVDDIARYQSELFEFIHASHQDLFDTILATKKLPEADKMNGALDAFAEQFQPTAAAAK

SEQ ID NO: 6 - DNA, 20 bp, Artificial Sequence
  Oligonucleotide primer
tcaaccagttgacggttcag

SEQ ID NO: 7 - DNA, 20 bp, Artificial Sequence
  Oligonucleotide primer
tttggttcaaaatggcatca